European Patent Application EP 4 599 843 A1, published August 13, 2025. Title: CAR AND MODIFIED CD200R COMBINATION. Applicant: Fundacio Institut de Recerca de la Santa Creu i Sant Pau. The sequence listing filed with the application follows.

SEQUENCE LISTING (44 sequences)

SEQ ID NO: 1 - protein, 595 aa, Homo sapiens
MRVLLAALGLLFLGALRAFPQDRPFEDTCHGNPSHYYDKAVRRCCYRCPMGLFPTQQCPQRPTDCRKQCEPDYYLDEADRCTACVTCSRDDLVEKTPCAWNSSRVCECRPGMFCSTSAVNSCARCFFHSVCPAGMIVKFPGTAQKNTVCEPASPGVSPACASPENCKEPSSGTIPQAKPTPVSPATSSASTMPVRGGTRLAQEAASKLTRAPDSPSSVGRPSSDPGLSPTQPCPEGSGDCRKQCEPDYYLDEAGRCTACVSCSRDDLVEKTPCAWNSSRTCECRPGMICATSATNSCARCVPYPICAAETVTKPQDMAEKDTTFEAPPLGTQPDCNPTPENGEAPASTSPTQSLLVDSQASKTLPIPTSAPVALSSTGKPVLDAGPVLFWVILVLVVVVGSSAFLLCHRRACRKRIRQKLHLCYPVQTSQPKLELVDSRPRRSSTQLRSGASVTEPVAEERGLMSQPLMETCHSVGAAYLESLPLQDASPAGGPSSPRDLPEPRVSTEHTNNKIEKIYIMKADTVIVGTVKAELPEGRGLAGPAEPELEEELEADHTPHYPEQETEPPLGSCSDVMLSVEEEGKEDPLPTAASGK

SEQ ID NO: 2 - protein, 254 aa, synthetic construct
QVTLKESGPGILQPSQTLSLTCSFSGFSLSTSGMGVSWIRQPSGKDLEWLAHIYWDDDKRYNPSLKSRLTISKDTSSNQVFLKITSVDTADTATYYCARRADGLYFYLDVWGAGTTVTVSSGSTSGSGKPGSGEGSTKGDIVMTQSQKFMSTSVGDRVSVTCKASQNVNTNVAWYQQKPGQSPEALIYSASYRYSGVPDRFTGSGSGTDFTLTISNVQSEDLAEYFCQQYNSYPLTFGSGTKLEIKRKAAAFVP

SEQ ID NO: 3 - protein, 530 aa, Homo sapiens
MRRLWGAARKPSGAGWEKEWAEAPQEAPGAWSGRLGPGRSGRKGRAVPGWASWPAHLALAARPARHLGGAGQGPRPLHSGTAPFHSRASGERQRRLEPQLQHESRCRSSTPADAWRAEAALPVRAMGAPWGSPTAAAGGRRGWRRGRGLPWTVCVLAAAGLTCTALITYACWGQLPPLPWASPTPSRPVGVLLWWEPFGGRDSAPRPPPDCRLRFNISGCRLLTDRASYGEAQAVLFHHRDLVKGPPDWPPPWGIQAHTAEEVDLRVLDYEEAAAAAEALATSSPRPPGQRWVWMNFESPSHSPGLRSLASNLFNWTLSYRADSDVFVPYGYLYPRSHPGDPPSGLAPPLSRKQGLVAWVVSHWDERQARVRYYHQLSQHVTVDVFGRGGPGQPVPEIGLLHTVARYKFYLAFENSQHLDYITEKLWRNALLAGAVPVVLGPDRANYERFVPRGAFIHVDDFPSASSLASYLLFLDRNPAVYRRYFHWRRSYAVHITSFWDEPWCRVCQAVQRAGDRPKSIRNLASWFER

SEQ ID NO: 4 - protein, 378 aa, Homo sapiens
MVLLWLTLLLIALPCLLQTKEDPNPPITNLRMKAKAQQLTWDLNRNVTDIECVKDADYSMPAVNNSYCQFGAISLCEVTNYTVRVANPPFSTWILFPENSGKPWAGAENLTCWIHDVDFLSCSWAVGPGAPADVQYDLYLNVANRRQQYECLHYKTDAQGTRIGCRFDDISRLSSGSQSSHILVRGRSAAFGIPCTDKFVVFSQIEILTPPNMTAKCNKTHSFMHWKMRSHFNRKFRYELQIQKRMQPVITEQVRDRTSFQLLNPGTYTVQIRARERVYEFLSAWSTPQRFECDQEEGANTRAWRTSLLIALGTLLALVCVFVICRRYLVMQRLFPRIPHMKDPIGDSFQNDKLVVWEAGKAGLEECLVTEVQVVQKT

SEQ ID NO: 5 - DNA, 762 bp, synthetic construct
  source 1..762: mol_type = other DNA
caggtgacactgaaggagtccggaccaggaatcctgcagccaagccagacactgtccctgacctgcagcttctccggcttttctctgagcacctccggcatgggcgtgtcctggatcaggcagccctctggcaaggatctggagtggctggcccacatctactgggacgatgacaagcggtacaatccttccctgaagtctcggctgacaatctctaaggacaccagctccaaccaggtgttcctgaagatcacaagcgtggataccgccgacacagccacctactattgcgcccggagagccgatggcctgtacttttatctggacgtgtggggagcaggaaccacagtgacagtgtctagcggatctaccagcggatccggcaagcctggatctggagagggcagcacaaagggcgatatcgtgatgacccagagccagaagttcatgtctacaagcgtgggcgacagagtgagcgtgacctgtaaggcctcccagaacgtgaatacaaacgtggcctggtaccagcagaagcctggccagagcccagaggccctgatctattccgcctcttacagatattccggcgtgccagataggttcacaggcagcggctccggcaccgactttacactgaccatctccaatgtgcagtctgaggacctggccgagtacttctgccagcagtacaactcttatccactgacatttggcagcggcaccaagctggagatcaagagaaaggcagcagccttcgtgcca

SEQ ID NO: 6 - protein, 164 aa, Homo sapiens
MKWKALFTAAILQAQLPITEAQSFGLLDPKLCYLLDGILFIYGVILTALFLRVKFSRSADAPAYQQGQNQLYNELNLGRREEYDVLDKRRGRDPEMGGKPQRRKNPQEGLYNELQKDKMAEAYSEIGMKGERRRGKGHDGLYQGLSTATKDTYDALHMQALPPR

SEQ ID NO: 7 - protein, 113 aa, synthetic construct
LRVKFSRSADAPAYKQGQNQLYNELNLGRREEYDVLDKRRGRDPEMGGKPRRKNPQEGLYNELQKDKMAEAYSEIGMKGERRRGKGHDGLYQGLSTATKDTYDALHMQALPPR

SEQ ID NO: 8 - RNA, 1600 nt, Homo sapiens
  source 1..1600: mol_type = mRNA
aaccgtcccggccaccgctgcctcagcctctgcctcccagcctctttctgagggaaaggacaagatgaagtggaaggcgcttttcaccgcggccatcctgcaggcacagttgccgattacagaggcacagagctttggcctgctggatcccaaactctgctacctgctggatggaatcctcttcatctatggtgtcattctcactgccttgttcctgagagtgaagttcagcaggagcgcagacgcccccgcgtaccagcagggccagaaccagctctataacgagctcaatctaggacgaagagaggagtacgatgttttggacaagagacgtggccgggaccctgagatggggggaaagccgcagagaaggaagaaccctcaggaaggcctgtacaatgaactgcagaaagataagatggcggaggcctacagtgagattgggatgaaaggcgagcgccggaggggcaaggggcacgatggcctttaccagggtctcagtacagccaccaaggacacctacgacgcccttcacatgcaggccctgccccctcgctaacagccaggggatttcaccactcaaaggccagacctgcagacgcccagattatgagacacaggatgaagcatttacaacccggttcactcttctcagccactgaagtattcccctttatgtacaggatgctttggttatatttagctccaaaccttcacacacagactgttgtccctgcactctttaagggagtgtactcccagggcttacggccctggccttgggccctctggtttgccggtggtgcaggtagacctgtctcctggcggttcctcgttctccctgggaggcgggcgcactgcctctcacagctgagttgttgagtctgttttgtaaagtccccagagaaagcgcagatgctagcacatgccctaatgtctgtatcactctgtgtctgagtggcttcactcctgctgtaaatttggcttctgttgtcaccttcacctcctttcaaggtaactgtactgggccatgttgtgcctccctggtgagagggccgggcagaggggcagatggaaaggagcctaggccaggtgcaaccagggagctgcaggggcatgggaaggtgggcgggcaggggagggtcagccagggcctgcgagggcagcgggagcctccctgcctcaggcctctgtgccgcaccattgaactgtaccatgtgctacaggggccagaagatgaacagactgaccttgatgagctgtgcacaaagtggcataaaaaacatgtggttacacagtgtgaataaagtgctgcggagcaagaggaggccgttgattcacttcacgctttcagcgaatgacaaaatcatctttgtgaaggcctcgcaggaagacccaacacatgggacctataactgcccagcggacagtggcaggacaggaaaaacccgtcaatgtactaggatactgctgcgtcattacagggcacaggccatggatggaaaacgctctctactctgctttttttctactgttttaatttatactggcatgctaaagccttcctattttgcataataaatgcttcagtgaaaatgca

SEQ ID NO: 9 - DNA, 339 bp, synthetic construct
  source 1..339: mol_type = other DNA
ctgagggtgaagttttctcggagcgccgacgcaccagcatacaagcagggacagaatcagctgtataatgagctgaacctgggcaggcgcgaggagtacgatgtgctggacaagaggagaggaagggatccagagatgggaggcaagcctaggcgcaagaatccacaggagggcctgtacaacgagctgcagaaggataagatggccgaggcctattccgagatcggcatgaagggagagcggagaaggggcaagggacacgacggactgtaccagggactgtctacagccaccaaggatacctatgacgcactgcacatgcaggccctgccaccaaga

SEQ ID NO: 10 - protein, 255 aa, Homo sapiens
MGNSCYNIVATLLLVLNFERTRSLQDPCSNCPAGTFCDNNRNQICSPCPPNSFSSAGGQRTCDICRQCKGVFRTRKECSSTSNAECDCTPGFHCLGAGCSMCEQDCKQGQELTKKGCKDCCFGTFNDQKRGICRPWTNCSLDGKSVLVNGTKERDVVCGPSPADLSPGASSVTPPAPAREPGHSPQIISFFLALTSTALLFLLFFLTLRFSVVKRGRKKLLYIFKQPFMRPVQTTQEEDGCSCRFPEEEEGGCEL

SEQ ID NO: 11 - RNA, 5872 nt, Homo sapiens
  source 1..5872: mol_type = mRNA
gcagaagcctgaagaccaaggagtggaaagttctccggcagccctgagatctcaagagtgacatttgtgagaccagctaatttgattaaaattctcttggaatcagctttgctagtatcatacctgtgccagatttcatcatgggaaacagctgttacaacatagtagccactctgttgctggtcctcaactttgagaggacaagatcattgcaggatccttgtagtaactgcccagctggtacattctgtgataataacaggaatcagatttgcagtccctgtcctccaaatagtttctccagcgcaggtggacaaaggacctgtgacatatgcaggcagtgtaaaggtgttttcaggaccaggaaggagtgttcctccaccagcaatgcagagtgtgactgcactccagggtttcactgcctgggggcaggatgcagcatgtgtgaacaggattgtaaacaaggtcaagaactgacaaaaaaaggttgtaaagactgttgctttgggacatttaacgatcagaaacgtggcatctgtcgaccctggacaaactgttctttggatggaaagtctgtgcttgtgaatgggacgaaggagagggacgtggtctgtggaccatctccagccgacctctctccgggagcatcctctgtgaccccgcctgcccctgcgagagagccaggacactctccgcagatcatctccttctttcttgcgctgacgtcgactgcgttgctcttcctgctgttcttcctcacgctccgtttctctgttgttaaacggggcagaaagaaactcctgtatatattcaaacaaccatttatgagaccagtacaaactactcaagaggaagatggctgtagctgccgatttccagaagaagaagaaggaggatgtgaactgtgaaatggaagtcaatagggctgttgggactttcttgaaaagaagcaaggaaatatgagtcatccgctatcacagctttcaaaagcaagaacaccatcctacataatacccaggattcccccaacacacgttcttttctaaatgccaatgagttggcctttaaaaatgcaccactttttttttttttttgacagggtctcactctgtcacccaggctggagtgcagtggcaccaccatggctctctgcagccttgacctctgggagctcaagtgatcctcctgcctcagtctcctgagtagctggaactacaaggaagggccaccacacctgactaacttttttgttttttgtttggtaaagatggcatttcaccatgttgtacaggctggtctcaaactcctaggttcactttggcctcccaaagtgctgggattacagacatgaactgccaggcccggccaaaataatgcaccacttttaacagaacagacagatgaggacagagctggtgataaaaaaaaaaaaaaaaaagcattttctagataccacttaacaggtttgagctagtttttttgaaatccaaagaaaattatagtttaaattcaattacatagtccagtggtccaactataattataatcaaaatcaatgcaggtttgttttttggtgctaatatgacatatgacaataagccacgaggtgcagtaagtacccgactaaagtttccgtgggttctgtcatgtaacacgacatgctccaccgtcaggggggagtatgagcagagtgcctgagtttagggtcaaggacaaaaaacctcaggcctggaggaagttttggaaagagttcaagtgtctgtatatcctatggtcttctccatcctcacaccttctgcctttgtcctgctcccttttaagccaggttacattctaaaaattcttaacttttaacataatattttataccaaagccaataaatgaactgcatatgataggtatgaagtacagtgagaaaattaacacctgtgagctcattgtcctaccacagcactagagtgggggccgccaaactcccatggccaaacctggtgcaccatttgcctttgtttgtctgttggtttgcttgagacagtcttgctctgttgcccaggctggaatggagtggctattcacaggcacaatcatagcacactttagccttaaactcctgggctcaagtgatccacccgcctcagtctcccaagtagctgggattacaggtgcaaacctggcatgcctgccattgtttggcttatgatctaaggatagctttttaaattttattcattttatttttttttgagacagtgtctcactctgtctcccaggctggagtacagtggtacaatcttggatcaccgcctcccagtttcaagtgatctccctgcctcagcctcctaagtagctgggactacaggtatgtgccaccacgcctggctaatttttatatttttagtagagacggggtttcaccatgttgtccaggctggtctcaaactcctgacctcaggtgatctgcccacctctgcctcccaaagtgctgggattacaggcatgagccaccatgcctggccatttcttacacttttgtatgacatgcctattgcaagcttgcgtgcctctgtcccatgttattttactctgggatttaggtggagggagcagcttctatttggaacattggccatcgcatggcaaatgggtatctgtcacttctgctcctatttagttggttctactataacctttagagcaaatcctgcagccaagccaggcatcaatagggcagaaaagtatattctgtaaataggggtgaggagaagatatttctgaacaatagtctactgcagtaccaaattgcttttcaaagtggctgttctaatgtactcccgtcagtcatataagtgtcatgtaagtatcccattgatccacatccttgctaccctctggtactatcaggtgcccttaattttgccaagccagtgggtatagaatgagatctcactgtggtcttagtttgcatttgcttggttactgatgagcaccttgtcaaatatttatataccatttgtgtttatttttttaaataaaatgcttgctcatgcttttttgcccatttgcaaaaaaacttggggccgggtgcagtggctcatgcctgtagtcccagctctttgggaggccaaggtgggcagatcgcttgagcccaggagttcgagaccagccttggcaacatggcgaaaccctgtctttacaaaaaatacaaaaattagccgggtgtggtggtgtgcacctgaagtcccagctactcagtaggttcgctttgagcctgggaggcagaggttgcagtgagctgggaccgcatcactacacttcagcctgggcaacagagaaaaaccttttctcagaaacaaacaaacccaaatgtggttgtttgtcctgattcctaaaaggtctttatgtattctagataataatctttggtcagttatatgtgttaaaaaatatcttctttgtggccaggcacggtagctcacacctgtaatcccagcactttgcggggctgaggtgggtggatcatctgaggtcaagagttcaagatcagcctggccaacacagtgaaaccccatctctactaaacatgtacaaaacttagctgggtatggtggcgggtgcctgtaaccccagctgctccagaggctgtggcagaagaatcgcttgaacccaggaggcagaggttgcagcgagccaagattgtgccattgcactccagactgggtgacaagagtgaaattctgcctatctatctatctatctatctatatctatatatatatatatatatatcctttgtaatttatttttccctttttaaaattttttataaaattcttttttatttttatttttagcagaggtgaggtttctgaggtttcattatgttgcccaggctggtcttgaactcctgagctcaagtgatcctcccacctcagccttccaaagtgctggaattgcagacatgagccaccgcgcccctcctgtttttctctaattaatggtgtctttctttgtctttctggtaataagcaaaaagttcttcatttgatttggttaaatttataactgttttctcatatggttaacattttttcttgcctggctaaagaaatccttttctgcccaatactataaagaggtttgcccacattttattccaaaagttttaagttttgtctttcatcttgaagtctaatgtatcaggaactggcttttgtgcctgttgggaggtagtgatccaattccatgtcttgcatgtaggtaaccactggtccctgcgccatgtattcaatacgtcgtctttctcctgcgggtctgcaatctcacctaccatccatcaagtttccatagggccatgggtctgcttctgggctccctgttctgttccattgtcaatttgtctatcctgtgccagtatcacactgtgtttattacaatagctttgtaacagctctcgatatccggtaggacatctccctccaccttctttttctacttcagaagtgtcttagctaggtcaggcacggtggctcacgcctgtaatcccagcactttgggaggccgacgcggatggatcacctgaggtcaggagttttgagacagcctggccaacatggtgaaaccccatctctactaaaaaatacaaaaattagtcaggcatggtggcatgtgcctgtaatcccagctatttgggaggctgaggccggagaattgcttgaacccggggggcggaggttgcagtgagccgagatcgtaccattgcactccagcctgggtgacagagcgaaactctgtctcaggaaaaaaaagaaaagagatgtcttggttattcttggttctttattattcaatataaattttagaagctgaatttgaaaagatttggattggaatttcattaaatctacaggtcaatttagggagagttgataattttacagaattgagtcatctggtgttccaataagaataagagaacaattattggctgtacaattcttgccaaatagtaggcaaagcaaagcttaggaagtatactggtgccatttcaggaacaaagctaggtgcgaatatttttgtctttctgaatcatgatgctgtaagttctaaagtgatttctcctcttggctttggacacatggtgtttaattacctactgctgactatccacaaacagaaagagactggtcatgccccacagggttggggtatccaagataatggagcgaggctctcatgtgtcctaggttacacaccgaaaatccacagtttattctgtgaagaaaggaggctatgtttatgatacagactgtgatatttttatcatagcctattctggtatcatgtgcaaaagctataaatgaaaaacacaggaacttggcatgtgagtcattgctccccctaaatgacaattaataaggaaggaacattgagacagaataaaatgatccccttctgggtttaatttagaaagttccataattaggtttaatagaaataaatgtaaatttctatgattaaaaataaattagcacatttagggatacacaaattataaatcattttctaaatgctaaaaacaagctcaggtttttttcagaagaaagttttaattttttttctttagtggaagatatcactctgacggaaagttttgatgtgaggggcggatgactataaagtgggcatcttcccccacaggaagatgtttccatctgtgggtgagaggtgcccaccgcagctagggcaggttacatgtgccctgtgtgtggtaggacttggagagtgatctttatcaacgtttttatttaaaagactatctaataaaacacaaaactatgatgttcacaggaaaaaaagaataagaaaaaaaga

SEQ ID NO: 12 - DNA, 126 bp, synthetic construct
  source 1..126: mol_type = other DNA
aagagaggcaggaagaagctgctgtatatcttcaagcagccctttatgcgccctgtgcagacaacccaggaggaggatggctgcagctgtcggttccctgaggaggaggagggaggatgtgagctg

SEQ ID NO: 13 - protein, 220 aa, Homo sapiens
MLRLLLALNLFPSIQVTGNKILVKQSPMLVAYDNAVNLSCKYSYNLFSREFRASLHKGLDSAVEVCVVYGNYSQQLQVYSKTGFNCDGKLGNESVTFYLQNLYVNQTDIYFCKIEVMYPPPYLDNEKSNGTIIHVKGKHLCPSPLFPGPSKPFWVLVVVGGVLACYSLLVTVAFIIFWVRSKRSRLLHSDYMNMTPRRPGPTRKHYQPYAPPRDFAAYRS

SEQ ID NO: 14 - RNA, 4721 nt, Homo sapiens
  source 1..4721: mol_type = mRNA
acacttcgggttcctcggggaggaggggctggaaccctagcccatcgtcaggacaaagatgctcaggctgctcttggctctcaacttattcccttcaattcaagtaacaggaaacaagattttggtgaagcagtcgcccatgcttgtagcgtacgacaatgcggtcaaccttagctgcaagtattcctacaatctcttctcaagggagttccgggcatcccttcacaaaggactggatagtgctgtggaagtctgtgttgtatatgggaattactcccagcagcttcaggtttactcaaaaacggggttcaactgtgatgggaaattgggcaatgaatcagtgacattctacctccagaatttgtatgttaaccaaacagatatttacttctgcaaaattgaagttatgtatcctcctccttacctagacaatgagaagagcaatggaaccattatccatgtgaaagggaaacacctttgtccaagtcccctatttcccggaccttctaagcccttttgggtgctggtggtggttggtggagtcctggcttgctatagcttgctagtaacagtggcctttattattttctgggtgaggagtaagaggagcaggctcctgcacagtgactacatgaacatgactccccgccgccccgggcccacccgcaagcattaccagccctatgccccaccacgcgacttcgcagcctatcgctcctgacacggacgcctatccagaagccagccggctggcagcccccatctgctcaatatcactgctctggataggaaatgaccgccatctccagccggccacctcaggcccctgttgggccaccaatgccaatttttctcgagtgactagaccaaatatcaagatcattttgagactctgaaatgaagtaaaagagatttcctgtgacaggccaagtcttacagtgccatggcccacattccaacttaccatgtacttagtgacttgactgagaagttagggtagaaaacaaaaagggagtggattctgggagcctcttccctttctcactcacctgcacatctcagtcaagcaaagtgtggtatccacagacattttagttgcagaagaaaggctaggaaatcattccttttggttaaatgggtgtttaatcttttggttagtgggttaaacggggtaagttagagtagggggagggataggaagacatatttaaaaaccattaaaacactgtctcccactcatgaaatgagccacgtagttcctatttaatgctgttttcctttagtttagaaatacatagacattgtcttttatgaattctgatcatatttagtcattttgaccaaatgagggatttggtcaaatgagggattccctcaaagcaatatcaggtaaaccaagttgctttcctcactccctgtcatgagacttcagtgttaatgttcacaatatactttcgaaagaataaaatagttctcctacatgaagaaagaatatgtcaggaaataaggtcactttatgtcaaaattatttgagtactatgggacctggcgcagtggctcatgcttgtaatcccagcactttgggaggccgaggtgggcagatcacttgagatcaggaccagcctggtcaagatggtgaaactccgtctgtactaaaaatacaaaatttagcttggcctggtggcaggcacctgtaatcccagctgcccaagaggctgaggcatgagaatcgcttgaacctggcaggcggaggttgcagtgagccgagatagtgccacagctctccagcctgggcgacagagtgagactccatctcaaacaacaacaacaacaacaacaacaacaacaaaccacaaaattatttgagtactgtgaaggattatttgtctaacagttcattccaatcagaccaggtaggagctttcctgtttcatatgtttcagggttgcacagttggtctctttaatgtcggtgtggagatccaaagtgggttgtggaaagagcgtccataggagaagtgagaatactgtgaaaaagggatgttagcattcattagagtatgaggatgagtcccaagaaggttctttggaaggaggacgaatagaatggagtaatgaaattcttgccatgtgctgaggagatagccagcattaggtgacaatcttccagaagtggtcaggcagaaggtgccctggtgagagctcctttacagggactttatgtggtttagggctcagagctccaaaactctgggctcagctgctcctgtaccttggaggtccattcacatgggaaagtattttggaatgtgtcttttgaagagagcatcagagttcttaagggactgggtaaggcctgaccctgaaatgaccatggatatttttctacctacagtttgagtcaactagaatatgcctggggaccttgaagaatggcccttcagtggccctcaccatttgttcatgcttcagttaattcaggtgttgaaggagcttaggttttagaggcacgtagacttggttcaagtctcgttagtagttgaatagcctcaggcaagtcactgcccacctaagatgatggttcttcaactataaaatggagataatggttacaaatgtctcttcctatagtataatctccataagggcatggcccaagtctgtctttgactctgcctatccctgacatttagtagcatgcccgacatacaatgttagctattggtattattgccatatagataaattatgtataaaaattaaactgggcaatagcctaagaaggggggaatattgtaacacaaatttaaacccactacgcagggatgaggtgctataatatgaggaccttttaacttccatcattttcctgtttcttgaaatagtttatcttgtaatgaaatataaggcacctcccacttttatgtatagaaagaggtcttttaatttttttttaatgtgagaaggaagggaggagtaggaatcttgagattccagatcgaaaatactgtactttggttgatttttaagtgggcttccattccatggatttaatcagtcccaagaagatcaaactcagcagtacttgggtgctgaagaactgttggatttaccctggcacgtgtgccacttgccagcttcttgggcacacagagttcttcaatccaagttatcagattgtatttgaaaatgacagagctggagagttttttgaaatggcagtggcaaataaataaatacttttttttaaatggaaagacttgatctatggtaataaatgattttgttttctgactggaaaaataggcctactaaagatgaatcacacttgagatgtttcttactcactctgcacagaaacaaagaagaaatgttatacagggaagtccgttttcactattagtatgaaccaagaaatggttcaaaaacagtggtaggagcaatgctttcatagtttcagatatggtagttatgaagaaaacaatgtcatttgctgctattattgtaagagtcttataattaatggtactcctataatttttgattgtgagctcacctatttgggttaagcatgccaatttaaagagaccaagtgtatgtacattatgttctacatattcagtgataaaattactaaactactatatgtctgctttaaatttgtactttaatattgtcttttggtattaagaaagatatgctttcagaatagatatgcttcgctttggcaaggaatttggatagaacttgctatttaaaagaggtgtggggtaaatccttgtataaatctccagtttagccttttttgaaaaagctagactttcaaatactaatttcacttcaagcagggtacgtttctggtttgtttgcttgacttcagtcacaatttcttatcagaccaatggctgacctctttgagatgtcaggctaggcttacctatgtgttctgtgtcatgtgaatgctgagaagtttgacagagatccaacttcagccttgaccccatcagtccctcgggttaactaactgagccaccggtcctcatggctattttaatgagggtattgatggttaaatgcatgtctgatcccttatcccagccatttgcactgccagctgggaactataccagacctggatactgatcccaaagtgttaaattcaactacatgctggagattagagatggtgccaataaaggacccagaaccaggatcttgattgctatagacttattaataatccaggtcaaagagagtgacacacactctctcaagacctggggtgagggagtctgtgttatctgcaaggccatttgaggctcagaaagtctctctttcctatagatatatgcatactttctgacatataggaatgtatcaggaatactcaaccatcacaggcatgttcctacctcagggcctttacatgtcctgtttactctgtctagaatgtccttctgtagatgacctggcttgcctcgtcacccttcaggtccttgctcaagtgtcatcttctcccctagttaaactaccccacaccctgtctgctttccttgcttatttttctccatagcattttaccatctcttacattagacatttttcttatttatttgtagtttataagcttcatgaggcaagtaactttgctttgtttcttgctgtatctccagtgcccagagcagtgcctggtatataataaatatttattgactgagtgaa

SEQ ID NO: 15 - protein, 154 aa, synthetic construct
KRGRKKLLYIFKQPFMRPVQTTQEEDGCSCRFPEEEEGGCELRVKFSRSADAPAYKQGQNQLYNELNLGRREEYDVLDKRRGRDPEMGGKPRRKNPQEGLYNELQKDKMAEAYSEIGMKGERRRGKGHDGLYQGLSTATKDTYDALHMQALPPR

SEQ ID NO: 16 - protein, 24 aa, Homo sapiens
IYIWAPLAGTCGVLLLSLVITLYC

SEQ ID NO: 17 - protein, 27 aa, Homo sapiens
FWVLVVVGGVLACYSLLVTVAFIIFWV

SEQ ID NO: 18 - protein, 21 aa, Homo sapiens
MALPVTALLLPLALLLHAARP

SEQ ID NO: 19 - protein, 69 aa, Homo sapiens
TTTPAPRPPTPAPTIASQPLSLRPEACRPAAGGAVHTRGLDFACDIYIWAPLAGTCGVLLLSLVITLYC

SEQ ID NO: 20 - protein, 39 aa, Homo sapiens
IEVMYPPPYLDNEKSNGTIIHVKGKHLCPSPLFPGPSKP

SEQ ID NO: 21 - protein, 498 aa, synthetic construct
MALPVTALLLPLALLLHAARPQVTLKESGPGILQPSQTLSLTCSFSGFSLSTSGMGVSWIRQPSGKDLEWLAHIYWDDDKRYNPSLKSRLTISKDTSSNQVFLKITSVDTADTATYYCARRADGLYFYLDVWGAGTTVTVSSGSTSGSGKPGSGEGSTKGDIVMTQSQKFMSTSVGDRVSVTCKASQNVNTNVAWYQQKPGQSPEALIYSASYRYSGVPDRFTGSGSGTDFTLTISNVQSEDLAEYFCQQYNSYPLTFGSGTKLEIKRKAAAFVPTTTPAPRPPTPAPTIASQPLSLRPEACRPAAGGAVHTRGLDFACDIYIWAPLAGTCGVLLLSLVITLYCKRGRKKLLYIFKQPFMRPVQTTQEEDGCSCRFPEEEEGGCELRVKFSRSADAPAYKQGQNQLYNELNLGRREEYDVLDKRRGRDPEMGGKPRRKNPQEGLYNELQKDKMAEAYSEIGMKGERRRGKGHDGLYQGLSTATKDTYDALHMQALPPR

SEQ ID NO: 22 - DNA, 1494 bp, synthetic construct
  source 1..1494: mol_type = other DNA
atggcactgccagtgaccgccctgctgctgcctctggccctgctgctgcacgcagcaagaccacaggtgacactgaaggagtccggaccaggaatcctgcagccaagccagacactgtccctgacctgcagcttctccggcttttctctgagcacctccggcatgggcgtgtcctggatcaggcagccctctggcaaggatctggagtggctggcccacatctactgggacgatgacaagcggtacaatccttccctgaagtctcggctgacaatctctaaggacaccagctccaaccaggtgttcctgaagatcacaagcgtggataccgccgacacagccacctactattgcgcccggagagccgatggcctgtacttttatctggacgtgtggggagcaggaaccacagtgacagtgtctagcggatctaccagcggatccggcaagcctggatctggagagggcagcacaaagggcgatatcgtgatgacccagagccagaagttcatgtctacaagcgtgggcgacagagtgagcgtgacctgtaaggcctcccagaacgtgaatacaaacgtggcctggtaccagcagaagcctggccagagcccagaggccctgatctattccgcctcttacagatattccggcgtgccagataggttcacaggcagcggctccggcaccgactttacactgaccatctccaatgtgcagtctgaggacctggccgagtacttctgccagcagtacaactcttatccactgacatttggcagcggcaccaagctggagatcaagagaaaggcagcagccttcgtgccaaccacaaccccagcaccaaggccacctacacctgcaccaaccatcgccagccagcctctgtccctgagaccagaggcctgtaggccagcagcaggaggagcagtgcacacccgcggcctggattttgcctgcgacatctatatctgggcacctctggccggaacctgtggcgtgctgctgctgtccctggtcatcaccctgtactgcaagagaggcaggaagaagctgctgtatatcttcaagcagccctttatgcgccctgtgcagacaacccaggaggaggatggctgcagctgtcggttccctgaggaggaggagggaggatgtgagctgagggtgaagttttctcggagcgccgacgcaccagcatacaagcagggacagaatcagctgtataatgagctgaacctgggcaggcgcgaggagtacgatgtgctggacaagaggagaggaagggatccagagatgggaggcaagcctaggcgcaagaatccacaggagggcctgtacaacgagctgcagaaggataagatggccgaggcctattccgagatcggcatgaagggagagcggagaaggggcaagggacacgacggactgtaccagggactgtctacagccaccaaggatacctatgacgcactgcacatgcaggccctgccaccaaga

SEQ ID NO: 23 - protein, 234 aa, synthetic construct
MLCPWRTANLGLLLILTIFLVAASSSLCMDEKQITQNYSKVLAEVNTSWPVKMATNAVLCCPPIALRNLIIITWEIILRGQPSCTKAYRKETNETKETNCTDERITWVSRPDQNSDLQIRPVAITHDGYYRCIMVTPDGNFHRGYHLQVLVTPEVTLFQNRNRTAVCKAVAGKPAAQISWIPEGDCATKQEYWSNGTVTVKSTCHWEVHNVSTVTCHVSHLTGNKSLYIELLPV

SEQ ID NO: 24 - DNA, 702 bp, synthetic construct
  source 1..702: mol_type = other DNA
atgctgtgcccttggagaaccgccaacctgggcctgctgctgatcctgaccatcttcctggtggccgccagcagcagcctgtgcatggacgagaagcagatcacccagaactacagcaaggtgctggccgaagtgaacaccagctggcccgtgaagatggccaccaacgccgtgctgtgctgccctcctatcgccctgcggaacctgatcatcatcacctgggagatcatcctgcggggccagcccagctgtaccaaggcctaccggaaagagacaaacgagacaaaagaaacaaactgcaccgacgagcggatcacatgggtgtccagacccgaccagaacagcgacctgcagatcagacccgtggccatcacccacgacggctactaccggtgcatcatggtcacccccgatggcaacttccaccggggataccatctgcaggtgctcgtgacccccgaagtgaccctgttccagaaccggaacagaaccgccgtgtgcaaggccgtggccggaaaacctgccgcccagatctcttggatccccgagggcgattgcgccaccaagcaggaatactggtccaacggcaccgtgaccgtgaagtccacctgtcactgggaggtgcacaacgtgtccaccgtgacatgccacgtgtcccacctgaccggcaacaagagcctgtacatcgagctgctgcctgtg

SEQ ID NO: 25 - DNA, 819 bp, synthetic construct
  source 1..819: mol_type = other DNA
atgctgtgcccttggaggaccgcaaacctgggactgctgctgatcctgacaatcttcctggtggccgccagctcctctctgtgcatggacgagaagcagatcacccagaactactctaaggtgctggccgaagtgaataccagctggccagtgaagatggccacaaacgccgtgctgtgctgtccccctatcgccctgaggaatctgatcatcatcacctgggagatcatcctgaggggccagcccagctgcacaaaggcctatcgcaaggagaccaacgagacaaaggagaccaattgtacagatgagaggatcacctgggtgtctcgccccgaccagaacagcgatctgcagatccggcctgtggccatcacccacgacggctactatagatgcatcatggtgacacccgatggcaatttccaccggggctaccacctgcaggtgctggtgacccctgaggtgacactgtttcagaacaggaataggaccgccgtgtgcaaggcagtggcaggcaagcctgcagcacagatctcctggatcccagagggcgactgtgccaccaagcaggagtactggagcaacggcaccgtgacagtgaagtccacatgccactgggaggtgcacaacgtgtccaccgtgacatgtcacgtgtctcacctgaccggcaataagagcctgtatatcgagctgctgcccgtgtgcccttccccactgttcccaggcccttctaagccattttgggtgctggtggtggtgggaggcgtgctggcctgttactccctgctggtgacagtggccttcatcatcttttgggtg

SEQ ID NO: 26 - protein, 21 aa, Homo sapiens
YIPYIILTIIILTIVGFIWLL

SEQ ID NO: 27 - protein, 12 aa, Homo sapiens
CPSPLFPGPSKP

SEQ ID NO: 28 - protein, 41 aa, Homo sapiens
RSKRSRLLHSDYMNMTPRRPGPTRKHYQPYAPPRDFAAYRS

SEQ ID NO: 29 - protein, 314 aa, synthetic construct
MLCPWRTANLGLLLILTIFLVAASSSLCMDEKQITQNYSKVLAEVNTSWPVKMATNAVLCCPPIALRNLIIITWEIILRGQPSCTKAYRKETNETKETNCTDERITWVSRPDQNSDLQIRPVAITHDGYYRCIMVTPDGNFHRGYHLQVLVTPEVTLFQNRNRTAVCKAVAGKPAAQISWIPEGDCATKQEYWSNGTVTVKSTCHWEVHNVSTVTCHVSHLTGNKSLYIELLPVCPSPLFPGPSKPFWVLVVVGGVLACYSLLVTVAFIIFWVRSKRSRLLHSDYMNMTPRRPGPTRKHYQPYAPPRDFAAYRS

SEQ ID NO: 30 - DNA, 942 bp, synthetic construct
  source 1..942: mol_type = other DNA
atgctgtgcccttggaggaccgcaaacctgggactgctgctgatcctgacaatcttcctggtggccgccagctcctctctgtgcatggacgagaagcagatcacccagaactactctaaggtgctggccgaagtgaataccagctggccagtgaagatggccacaaacgccgtgctgtgctgtccccctatcgccctgaggaatctgatcatcatcacctgggagatcatcctgaggggccagcccagctgcacaaaggcctatcgcaaggagaccaacgagacaaaggagaccaattgtacagatgagaggatcacctgggtgtctcgccccgaccagaacagcgatctgcagatccggcctgtggccatcacccacgacggctactatagatgcatcatggtgacacccgatggcaatttccaccggggctaccacctgcaggtgctggtgacccctgaggtgacactgtttcagaacaggaataggaccgccgtgtgcaaggcagtggcaggcaagcctgcagcacagatctcctggatcccagagggcgactgtgccaccaagcaggagtactggagcaacggcaccgtgacagtgaagtccacatgccactgggaggtgcacaacgtgtccaccgtgacatgtcacgtgtctcacctgaccggcaataagagcctgtatatcgagctgctgcccgtgtgcccttccccactgttcccaggcccttctaagccattttgggtgctggtggtggtgggaggcgtgctggcctgttactccctgctggtgacagtggccttcatcatcttttgggtgaggagcaagcggtccagactgctgcactctgactatatgaatatgaccccacggagaccaggaccaacaaggaagcactaccagccctatgccccaccccgggattttgccgcctatagaagc

SEQ ID NO: 31 - DNA, 2511 bp, synthetic construct
  source 1..2511: mol_type = other DNA
atggcactgccagtgaccgccctgctgctgcctctggccctgctgctgcacgcagcaagaccacaggtgacactgaaggagtccggaccaggaatcctgcagccaagccagacactgtccctgacctgcagcttctccggcttttctctgagcacctccggcatgggcgtgtcctggatcaggcagccctctggcaaggatctggagtggctggcccacatctactgggacgatgacaagcggtacaatccttccctgaagtctcggctgacaatctctaaggacaccagctccaaccaggtgttcctgaagatcacaagcgtggataccgccgacacagccacctactattgcgcccggagagccgatggcctgtacttttatctggacgtgtggggagcaggaaccacagtgacagtgtctagcggatctaccagcggatccggcaagcctggatctggagagggcagcacaaagggcgatatcgtgatgacccagagccagaagttcatgtctacaagcgtgggcgacagagtgagcgtgacctgtaaggcctcccagaacgtgaatacaaacgtggcctggtaccagcagaagcctggccagagcccagaggccctgatctattccgcctcttacagatattccggcgtgccagataggttcacaggcagcggctccggcaccgactttacactgaccatctccaatgtgcagtctgaggacctggccgagtacttctgccagcagtacaactcttatccactgacatttggcagcggcaccaagctggagatcaagagaaaggcagcagccttcgtgccaaccacaaccccagcaccaaggccacctacacctgcaccaaccatcgccagccagcctctgtccctgagaccagaggcctgtaggccagcagcaggaggagcagtgcacacccgcggcctggattttgcctgcgacatctatatctgggcacctctggccggaacctgtggcgtgctgctgctgtccctggtcatcaccctgtactgcaagagaggcaggaagaagctgctgtatatcttcaagcagccctttatgcgccctgtgcagacaacccaggaggaggatggctgcagctgtcggttccctgaggaggaggagggaggatgtgagctgagggtgaagttttctcggagcgccgacgcaccagcatacaagcagggacagaatcagctgtataatgagctgaacctgggcaggcgcgaggagtacgatgtgctggacaagaggagaggaagggatccagagatgggaggcaagcctaggcgcaagaatccacaggagggcctgtacaacgagctgcagaaggataagatggccgaggcctattccgagatcggcatgaagggagagcggagaaggggcaagggacacgacggactgtaccagggactgtctacagccaccaaggatacctatgacgcactgcacatgcaggccctgccaccaagaatcgatctggagggcggaggagagggaaggggatccctgctgacatgcggcgacgtggaggagaatcccggccctatgctgtgcccttggaggaccgcaaacctgggactgctgctgatcctgacaatcttcctggtggccgccagctcctctctgtgcatggacgagaagcagatcacccagaactactctaaggtgctggccgaagtgaataccagctggccagtgaagatggccacaaacgccgtgctgtgctgtccccctatcgccctgaggaatctgatcatcatcacctgggagatcatcctgaggggccagcccagctgcacaaaggcctatcgcaaggagaccaacgagacaaaggagaccaattgtacagatgagaggatcacctgggtgtctcgccccgaccagaacagcgatctgcagatccggcctgtggccatcacccacgacggctactatagatgcatcatggtgacacccgatggcaatttccaccggggctaccacctgcaggtgctggtgacccctgaggtgacactgtttcagaacaggaataggaccgccgtgtgcaaggcagtggcaggcaagcctgcagcacagatctcctggatcccagagggcgactgtgccaccaagcaggagtactggagcaacggcaccgtgacagtgaagtccacatgccactgggaggtgcacaacgtgtccaccgtgacatgtcacgtgtctcacctgaccggcaataagagcctgtatatcgagctgctgcccgtgtgcccttccccactgttcccaggcccttctaagccattttgggtgctggtggtggtgggaggcgtgctggcctgttactccctgctggtgacagtggccttcatcatcttttgggtgaggagcaagcggtccagactgctgcactctgactatatgaatatgaccccacggagaccaggaccaacaaggaagcactaccagccctatgccccaccccgggattttgccgcctatagaagc

SEQ ID NO: 32 - protein, 837 aa, synthetic construct
MALPVTALLLPLALLLHAARPQVTLKESGPGILQPSQTLSLTCSFSGFSLSTSGMGVSWIRQPSGKDLEWLAHIYWDDDKRYNPSLKSRLTISKDTSSNQVFLKITSVDTADTATYYCARRADGLYFYLDVWGAGTTVTVSSGSTSGSGKPGSGEGSTKGDIVMTQSQKFMSTSVGDRVSVTCKASQNVNTNVAWYQQKPGQSPEALIYSASYRYSGVPDRFTGSGSGTDFTLTISNVQSEDLAEYFCQQYNSYPLTFGSGTKLEIKRKAAAFVPTTTPAPRPPTPAPTIASQPLSLRPEACRPAAGGAVHTRGLDFACDIYIWAPLAGTCGVLLLSLVITLYCKRGRKKLLYIFKQPFMRPVQTTQEEDGCSCRFPEEEEGGCELRVKFSRSADAPAYKQGQNQLYNELNLGRREEYDVLDKRRGRDPEMGGKPRRKNPQEGLYNELQKDKMAEAYSEIGMKGERRRGKGHDGLYQGLSTATKDTYDALHMQALPPRIDLEGGGEGRGSLLTCGDVEENPGPMLCPWRTANLGLLLILTIFLVAASSSLCMDEKQITQNYSKVLAEVNTSWPVKMATNAVLCCPPIALRNLIIITWEIILRGQPSCTKAYRKETNETKETNCTDERITWVSRPDQNSDLQIRPVAITHDGYYRCIMVTPDGNFHRGYHLQVLVTPEVTLFQNRNRTAVCKAVAGKPAAQISWIPEGDCATKQEYWSNGTVTVKSTCHWEVHNVSTVTCHVSHLTGNKSLYIELLPVCPSPLFPGPSKPFWVLVVVGGVLACYSLLVTVAFIIFWVRSKRSRLLHSDYMNMTPRRPGPTRKHYQPYAPPRDFAAYRS

SEQ ID NO: 33 - DNA, 819 bp, synthetic construct; identical to SEQ ID NO: 25
  source 1..819: mol_type = other DNA

SEQ ID NO: 34 - protein, 273 aa, synthetic construct
MLCPWRTANLGLLLILTIFLVAASSSLCMDEKQITQNYSKVLAEVNTSWPVKMATNAVLCCPPIALRNLIIITWEIILRGQPSCTKAYRKETNETKETNCTDERITWVSRPDQNSDLQIRPVAITHDGYYRCIMVTPDGNFHRGYHLQVLVTPEVTLFQNRNRTAVCKAVAGKPAAQISWIPEGDCATKQEYWSNGTVTVKSTCHWEVHNVSTVTCHVSHLTGNKSLYIELLPVCPSPLFPGPSKPFWVLVVVGGVLACYSLLVTVAFIIFWV

SEQ ID NO: 35 - DNA, 2388 bp, synthetic construct
  source 1..2388: mol_type = other DNA
atggcactgccagtgaccgccctgctgctgcctctggccctgctgctgcacgcagcaagaccacaggtgacactgaaggagtccggaccaggaatcctgcagccaagccagacactgtccctgacctgcagcttctccggcttttctctgagcacctccggcatgggcgtgtcctggatcaggcagccctctggcaaggatctggagtggctggcccacatctactgggacgatgacaagcggtacaatccttccctgaagtctcggctgacaatctctaaggacaccagctccaaccaggtgttcctgaagatcacaagcgtggataccgccgacacagccacctactattgcgcccggagagccgatggcctgtacttttatctggacgtgtggggagcaggaaccacagtgacagtgtctagcggatctaccagcggatccggcaagcctggatctggagagggcagcacaaagggcgatatcgtgatgacccagagccagaagttcatgtctacaagcgtgggcgacagagtgagcgtgacctgtaaggcctcccagaacgtgaatacaaacgtggcctggtaccagcagaagcctggccagagcccagaggccctgatctattccgcctcttacagatattccggcgtgccagataggttcacaggcagcggctccggcaccgactttacactgaccatctccaatgtgcagtctgaggacctggccgagtacttctgccagcagtacaactcttatccactgacatttggcagcggcaccaagctggagatcaagagaaaggcagcagccttcgtgccaaccacaaccccagcaccaaggccacctacacctgcaccaaccatcgccagccagcctctgtccctgagaccagaggcctgtaggccagcagcaggaggagcagtgcacacccgcggcctggattttgcctgcgacatctatatctgggcacctctggccggaacctgtggcgtgctgctgctgtccctggtcatcaccctgtactgcaagagaggcaggaagaagctgctgtatatcttcaagcagccctttatgcgccctgtgcagacaacccaggaggaggatggctgcagctgtcggttccctgaggaggaggagggaggatgtgagctgagggtgaagttttctcggagcgccgacgcaccagcatacaagcagggacagaatcagctgtataatgagctgaacctgggcaggcgcgaggagtacgatgtgctggacaagaggagaggaagggatccagagatgggaggcaagcctaggcgcaagaatccacaggagggcctgtacaacgagctgcagaaggataagatggccgaggcctattccgagatcggcatgaagggagagcggagaaggggcaagggacacgacggactgtaccagggactgtctacagccaccaaggatacctatgacgcactgcacatgcaggccctgccaccaagaatcgatctggagggcggaggagagggaaggggatccctgctgacatgcggcgacgtggaggagaatcccggccctatgctgtgcccttggaggaccgcaaacctgggactgctgctgatcctgacaatcttcctggtggccgccagctcctctctgtgcatggacgagaagcagatcacccagaactactctaaggtgctggccgaagtgaataccagctggccagtgaagatggccacaaacgccgtgctgtgctgtccccctatcgccctgaggaatctgatcatcatcacctgggagatcatcctgaggggccagcccagctgcacaaaggcctatcgcaaggagaccaacgagacaaaggagaccaattgtacagatgagaggatcacctgggtgtctcgccccgaccagaacagcgatctgcagatccggcctgtggccatcacccacgacggctactatagatgcatcatggtgacacccgatggcaatttccaccggggctaccacctgcaggtgctggtgacccctgaggtgacactgtttcagaacaggaataggaccgccgtgtgcaaggcagtggcaggcaagcctgcagcacagatctcctggatcccagagggcgactgtgccaccaagcaggagtactggagcaacggcaccgtgacagtgaagtccacatgccactgggaggtgcacaacgtgtccaccgtgacatgtcacgtgtctcacctgaccggcaataagagcctgtatatcgagctgctgcccgtgtgcccttccccactgttcccaggcccttctaagccattttgggtgctggtggtggtgggaggcgtgctggcctgttactccctgctggtgacagtggccttcatcatcttttgggtg

SEQ ID NO: 36 - protein, 796 aa, synthetic construct
MALPVTALLLPLALLLHAARPQVTLKESGPGILQPSQTLSLTCSFSGFSLSTSGMGVSWIRQPSGKDLEWLAHIYWDDDKRYNPSLKSRLTISKDTSSNQVFLKITSVDTADTATYYCARRADGLYFYLDVWGAGTTVTVSSGSTSGSGKPGSGEGSTKGDIVMTQSQKFMSTSVGDRVSVTCKASQNVNTNVAWYQQKPGQSPEALIYSASYRYSGVPDRFTGSGSGTDFTLTISNVQSEDLAEYFCQQYNSYPLTFGSGTKLEIKRKAAAFVPTTTPAPRPPTPAPTIASQPLSLRPEACRPAAGGAVHTRGLDFACDIYIWAPLAGTCGVLLLSLVITLYCKRGRKKLLYIFKQPFMRPVQTTQEEDGCSCRFPEEEEGGCELRVKFSRSADAPAYKQGQNQLYNELNLGRREEYDVLDKRRGRDPEMGGKPRRKNPQEGLYNELQKDKMAEAYSEIGMKGERRRGKGHDGLYQGLSTATKDTYDALHMQALPPRIDLEGGGEGRGSLLTCGDVEENPGPMLCPWRTANLGLLLILTIFLVAASSSLCMDEKQITQNYSKVLAEVNTSWPVKMATNAVLCCPPIALRNLIIITWEIILRGQPSCTKAYRKETNETKETNCTDERITWVSRPDQNSDLQIRPVAITHDGYYRCIMVTPDGNFHRGYHLQVLVTPEVTLFQNRNRTAVCKAVAGKPAAQISWIPEGDCATKQEYWSNGTVTVKSTCHWEVHNVSTVTCHVSHLTGNKSLYIELLPVCPSPLFPGPSKPFWVLVVVGGVLACYSLLVTVAFIIFWV

SEQ ID NO: 37 - protein, 539 aa, synthetic construct
MALPVTALLLPLALLLHAARPQVTLKESGPGILQPSQTLSLTCSFSGFSLSTSGMGVSWIRQPSGKDLEWLAHIYWDDDKRYNPSLKSRLTISKDTSSNQVFLKITSVDTADTATYYCARRADGLYFYLDVWGAGTTVTVSSGSTSGSGKPGSGEGSTKGDIVMTQSQKFMSTSVGDRVSVTCKASQNVNTNVAWYQQKPGQSPEALIYSASYRYSGVPDRFTGSGSGTDFTLTISNVQSEDLAEYFCQQYNSYPLTFGSGTKLEIKRKAAAFVPTTTPAPRPPTPAPTIASQPLSLRPEACRPAAGGAVHTRGLDFACDIYIWAPLAGTCGVLLLSLVITLYCRSKRSRLLHSDYMNMTPRRPGPTRKHYQPYAPPRDFAAYRSKRGRKKLLYIFKQPFMRPVQTTQEEDGCSCRFPEEEEGGCELRVKFSRSADAPAYKQGQNQLYNELNLGRREEYDVLDKRRGRDPEMGGKPRRKNPQEGLYNELQKDKMAEAYSEIGMKGERRRGKGHDGLYQGLSTATKDTYDALHMQALPPR

SEQ ID NO: 38 - DNA, 1617 bp, synthetic construct
  source 1..1617: mol_type = other DNA
atggcactgccagtgaccgccctgctgctgcctctggccctgctgctgcacgcagcaagaccacaggtgacactgaaggagtccggaccaggaatcctgcagccaagccagacactgtccctgacctgcagcttctccggcttttctctgagcacctccggcatgggcgtgtcctggatcaggcagccctctggcaaggatctggagtggctggcccacatctactgggacgatgacaagcggtacaatccttccctgaagtctcggctgacaatctctaaggacaccagctccaaccaggtgttcctgaagatcacaagcgtggataccgccgacacagccacctactattgcgcccggagagccgatggcctgtacttttatctggacgtgtggggagcaggaaccacagtgacagtgtctagcggatctaccagcggatccggcaagcctggatctggagagggcagcacaaagggcgatatcgtgatgacccagagccagaagttcatgtctacaagcgtgggcgacagagtgagcgtgacctgtaaggcctcccagaacgtgaatacaaacgtggcctggtaccagcagaagcctggccagagcccagaggccctgatctattccgcctcttacagatattccggcgtgccagataggttcacaggcagcggctccggcaccgactttacactgaccatctccaatgtgcagtctgaggacctggccgagtacttctgccagcagtacaactcttatccactgacatttggcagcggcaccaagctggagatcaagagaaaggcagcagccttcgtgccaaccacaaccccagcaccaaggccacctacacctgcaccaaccatcgccagccagcctctgtccctgagaccagaggcctgtaggccagcagcaggaggagcagtgcacacccgcggcctggattttgcctgcgacatctatatctgggcacctctggccggaacctgtggcgtgctgctgctgtccctggtcatcaccctgtactgcaggagcaagcggtccagactgctgcactctgactatatgaatatgaccccacggagaccaggaccaacaaggaagcactaccagccctatgccccaccccgggattttgccgcctatagaagcaagagaggcaggaagaagctgctgtatatcttcaagcagccctttatgcgccctgtgcagacaacccaggaggaggatggctgcagctgtcggttccctgaggaggaggagggaggatgtgagctgagggtgaagttttctcggagcgccgacgcaccagcatacaagcagggacagaatcagctgtataatgagctgaacctgggcaggcgcgaggagtacgatgtgctggacaagaggagaggaagggatccagagatgggaggcaagcctaggcgcaagaatccacaggagggcctgtacaacgagctgcagaaggataagatggccgaggcctattccgagatcggcatgaagggagagcggagaaggggcaagggacacgacggactgtaccagggactgtctacagccaccaaggatacctatgacgcactgcacatgcaggccctgccaccaaga

SEQ ID NO: 39 - DNA, 1074 bp, synthetic construct
  source 1..1074: mol_type = other DNA
agaatgctgctgctcgtgacctctctgctgctgtgcgagctgccccaccctgcctttctgctgatcccccggaaagtgtgcaacggcatcggcatcggagagttcaaggactccctgagcatcaacgccaccaacatcaagcacttcaagaactgcaccagcatcagcggcgacctgcacatcctgcccgtggcctttagaggcgacagctttacccacacccccccactggaccctcaggaactggacatcctgaaaaccgtgaaagagatcaccggatttctgctgattcaggcctggcccgagaaccggacagacctgcacgccttcgagaacctggaaattatccggggcaggaccaagcagcacggccagttttctctggccgtggtgtccctgaacatcacctccctgggcctgcggagcctgaaagaaatctccgatggcgacgtgatcatctccggcaacaagaacctgtgctacgccaacaccatcaactggaagaagctgttcggcacctccggccagaaaactaagatcatcagcaaccggggcgagaacagctgcaaggccacaggacaagtgtgccacgccctgtgtagccctgagggctgttggggacccgagcccagagattgtgtgtcctgccggaacgtgtcccggggcagagaatgcgtggacaagtgcaacctgctggaaggcgagccccgcgagttcgtggaaaacagcgagtgcatccagtgccaccccgagtgtctgccccaggccatgaacattacctgcaccggcagaggccccgacaactgtatccagtgcgcccactacatcgacggcccccactgcgtgaaaacctgtccagctggcgtgatgggagagaacaataccctcgtgtggaagtatgccgacgccggccacgtgtgccacctgtgtcaccccaattgcacctacggctgtaccggccctggactggaaggctgcccaacaaacggccccaagatccccagcattgccaccggcatggtgggagccttgctgctgctgctggtggtggccctgggcatcggcctgttcatg

SEQ ID NO: 40 - protein, 358 aa, synthetic construct
RMLLLVTSLLLCELPHPAFLLIPRKVCNGIGIGEFKDSLSINATNIKHFKNCTSISGDLHILPVAFRGDSFTHTPPLDPQELDILKTVKEITGFLLIQAWPENRTDLHAFENLEIIRGRTKQHGQFSLAVVSLNITSLGLRSLKEISDGDVIISGNKNLCYANTINWKKLFGTSGQKTKIISNRGENSCKATGQVCHALCSPEGCWGPEPRDCVSCRNVSRGRECVDKCNLLEGEPREFVENSECIQCHPECLPQAMNITCTGRGPDNCIQCAHYIDGPHCVKTCPAGVMGENNTLVWKYADAGHVCHLCHPNCTYGCTGPGLEGCPTNGPKIPSIATGMVGALLLLLVVALGIGLFM

SEQ ID NO: 41 - DNA, 2643 bp, synthetic construct
  source 1..2643: mol_type = other DNA
atggctctgcctgtgacagctctgctgctgcctctggccctgctgctgcatgctgctagaccccaagtgaccctgaaagagagcggccctggcatcctgcagcctagccagacactgagcctgacctgcagcttcagcggcttcagcctgagcacaagcggcatgggcgtgtcctggatcagacagcccagcggcaaggacctggaatggctggcccacatctactgggacgacgacaagcggtacaaccccagcctgaagtcccggctgaccatcagcaaggacaccagcagcaaccaggtgttcctgaagatcacctccgtggacaccgccgataccgccacctactactgtgccagaagggccgacggcctgtacttctacctggacgtgtggggagccggcaccaccgtgacagtgtctagcggcagcacatccggctctggcaagcctggatctggcgagggcagcaccaagggcgacatcgtgatgacccagagccagaaattcatgagcaccagcgtgggcgaccgggtgtccgtgacatgtaaagccagccagaacgtgaacaccaacgtggcctggtatcagcagaagcccggccagtctcctgaggccctgatctacagcgccagctacagatacagcggcgtgcccgacagattcaccggcagcggcagcggaaccgacttcaccctgaccatctccaacgtgcagagcgaggacctggccgagtacttctgccagcagtacaacagctaccccctgaccttcggctccggcaccaagctggaaatcaagcggaaggccgctgccttcgtgcccacaacaacacccgctcctagaccccctacccctgcccctacaatcgccagccagcctctgtctctgcggcccgaagcttgtagaccagctgctggcggagccgtgcacaccagaggactggatttcgcctgcgacatctacatctgggcccctctggccggcacatgtggcgtgctgctgctgagcctcgtgatcaccctgtactgcaagcggggcagaaagaagctgctgtacatcttcaagcagcccttcatgcggcccgtgcagaccacccaggaagaggacggctgctcctgcagattccccgaggaagaagaaggcggctgcgagctgagagtgaagttcagcagatccgccgacgcccctgcctacaagcagggacagaaccagctgtacaatgagctgaacctgggcagacgggaagagtacgacgtgctggacaagcggagaggcagggaccctgagatgggcggcaagcccagaagaaagaacccccaggaaggcctgtataacgagctgcagaaagacaagatggccgaggcctacagcgagatcggaatgaagggcgagcggagaagaggcaagggccacgatggactgtaccagggcctgtccaccgccaccaaggatacctacgacgccctgcacatgcaggccctgccccccagaatcgatctggaaggcggcggagagggcagaggcagcctgctgacatgcggcgacgtggaagagaacccaggccccagaatgctgctgctcgtgacctctctgctgctgtgcgagctgccccaccctgcctttctgctgatcccccggaaagtgtgcaacggcatcggcatcggagagttcaaggactccctgagcatcaacgccaccaacatcaagcacttcaagaactgcaccagcatcagcggcgacctgcacatcctgcccgtggcctttagaggcgacagctttacccacacccccccactggaccctcaggaactggacatcctgaaaaccgtgaaagagatcaccggatttctgctgattcaggcctggcccgagaaccggacagacctgcacgccttcgagaacctggaaattatccggggcaggaccaagcagcacggccagttttctctggccgtggtgtccctgaacatcacctccctgggcctgcggagcctgaaagaaatctccgatggcgacgtgatcatctccggcaacaagaacctgtgctacgccaacaccatcaactggaagaagctgttcggcacctccggccagaaaactaagatcatcagcaaccggggcgagaacagctgcaaggccacaggacaagtgtgccacgccctgtgtagccctgagggctgttggggacccgagcccagagattgtgtgtcctgccggaacgtgtcccggggcagagaatgcgtggacaagtgcaacctgctggaaggcgagccccgcgagttcgtggaaaacagcgagtgcatccagtgccaccccgagtgtctgccccaggccatgaacattacctgcaccggcagaggccccgacaactgtatccagtgcgcccactacatcgacggcccccactgcgtgaaaacctgtccagctggcgtgatgggagagaacaataccctcgtgtggaagtatgccgacgccggccacgtgtgccacctgtgtcaccccaattgcacctacggctgtaccggccctggactggaaggctgcccaacaaacggccccaagatccccagcattgccaccggcatggtgggagccttgctgctgctgctggtggtggccctgggcatcggcctgttcatg

SEQ ID NO: 42 - protein, 881 aa, synthetic construct
MALPVTALLLPLALLLHAARPQVTLKESGPGILQPSQTLSLTCSFSGFSLSTSGMGVSWIRQPSGKDLEWLAHIYWDDDKRYNPSLKSRLTISKDTSSNQVFLKITSVDTADTATYYCARRADGLYFYLDVWGAGTTVTVSSGSTSGSGKPGSGEGSTKGDIVMTQSQKFMSTSVGDRVSVTCKASQNVNTNVAWYQQKPGQSPEALIYSASYRYSGVPDRFTGSGSGTDFTLTISNVQSEDLAEYFCQQYNSYPLTFGSGTKLEIKRKAAAFVPTTTPAPRPPTPAPTIASQPLSLRPEACRPAAGGAVHTRGLDFACDIYIWAPLAGTCGVLLLSLVITLYCKRGRKKLLYIFKQPFMRPVQTTQEEDGCSCRFPEEEEGGCELRVKFSRSADAPAYKQGQNQLYNELNLGRREEYDVLDKRRGRDPEMGGKPRRKNPQEGLYNELQKDKMAEAYSEIGMKGERRRGKGHDGLYQGLSTATKDTYDALHMQALPPRIDLEGGGEGRGSLLTCGDVEENPGPRMLLLVTSLLLCELPHPAFLLIPRKVCNGIGIGEFKDSLSINATNIKHFKNCTSISGDLHILPVAFRGDSFTHTPPLDPQELDILKTVKEITGFLLIQAWPENRTDLHAFENLEIIRGRTKQHGQFSLAVVSLNITSLGLRSLKEISDGDVIISGNKNLCYANTINWKKLFGTSGQKTKIISNRGENSCKATGQVCHALCSPEGCWGPEPRDCVSCRNVSRGRECVDKCNLLEGEPREFVENSECIQCHPECLPQAMNITCTGRGPDNCIQCAHYIDGPHCVKTCPAGVMGENNTLVWKYADAGHVCHLCHPNCTYGCTGPGLEGCPTNGPKIPSIATGMVGALLLLLVVALGIGLFM

SEQ ID NO: 43 - DNA, 2643 bp, synthetic construct; identical to SEQ ID NO: 41
  source 1..2643: mol_type = other DNA

SEQ ID NO: 44 - protein, 881 aa, synthetic construct; identical to SEQ ID NO: 42